European Patent Application EP 4 681 700 A1, published January 21, 2026. Title: GSE24.2 derived peptide and uses thereof. Applicant: CONSEJO SUPERIOR DE INVESTIGACIONES CIENTIFICAS. The sequence listing filed with the application follows.

SEQUENCE LISTING (64 sequences)

SEQ ID NO: 1 - protein, 10 aa, synthetic construct
DKPSNPSSHE

SEQ ID NO: 2 - protein, 11 aa, synthetic construct
GFINLDKPSNP

SEQ ID NO: 3 - protein, 55 aa, synthetic construct
GFINLDKPSNPSSHEVVAWIRRILRVEKTGHSGTLDPKVTGCLIVCIERATRLVK

SEQ ID NO: 4 - protein, 17 aa, synthetic construct
GFINLDKPSNPSSHEVV

SEQ ID NO: 5 - protein, 18 aa, synthetic construct
GFINLDKPSNPSSHEVVA

SEQ ID NO: 6 - protein, 19 aa, synthetic construct
GFINLDKPSNPSSHEVVAW

SEQ ID NO: 7 - protein, 25 aa, synthetic construct
GFINLDKPSNPSSHEVVAWIRRILR

SEQ ID NO: 8 - protein, 59 aa, synthetic construct
GFINLDKPSNPSSHEVVAWIRRILRVEKTGHSGTLDPKVTGCLIVCIERATRLVKKRKR

SEQ ID NO: 9 - protein, 63 aa, synthetic construct
GFINLDKPSNPSSHEVVAWIRRILRVEKTGHSGTLDPKVTGCLIVCIERATRLVKKKEKKKSK

SEQ ID NO: 10 - protein, 59 aa, synthetic construct
KRKRGFLNLDKPSNPSSHEVVAWIRRILRVEKTGHSGTLDPKVTGCLIVCIERATRLVK

SEQ ID NO: 11 - protein, 63 aa, synthetic construct
KKEKKKSKGFINLDKPSNPSSHEVVAWIRRILRVEKTGHSGTLDPKVTGCLIVCIERATRLVK

SEQ ID NO: 12 - protein, 8 aa, synthetic construct
NLDKPSNP

SEQ ID NO: 13 - protein, 12 aa, synthetic construct
NLDKPSNPSSHE

SEQ ID NO: 14 - protein, 7 aa, synthetic construct
GFINLDK

SEQ ID NO: 15 - protein, 6 aa, synthetic construct
DKPSNP

SEQ ID NO: 16 - protein, 10 aa, synthetic construct
EHSSPNSPKD

SEQ ID NO: 17 - protein, 14 aa, synthetic construct
DKPSNPSSHEKRKR

SEQ ID NO: 18 - protein, 18 aa, synthetic construct
DKPSNPSSHEKKEKKKSK

SEQ ID NO: 19 - protein, 4 aa, synthetic construct
KRKR

SEQ ID NO: 20 - protein, 8 aa, synthetic construct
KKEKKKSK

SEQ ID NO: 21 - DNA, 20 bp, synthetic construct
  source 1..20: mol_type = other DNA
cggaagagtgtctggagcaa

SEQ ID NO: 22 - DNA, 18 bp, synthetic construct
  source 1..18: mol_type = other DNA
ggatgaagcggagtctgg

SEQ ID NO: 23 - DNA, 20 bp, synthetic construct
  source 1..20: mol_type = other DNA
gagtgtcactaagggccaag

SEQ ID NO: 24 - DNA, 20 bp, synthetic construct
  source 1..20: mol_type = other DNA
cagctgcagtcttaaggagg

SEQ ID NO: 25 - DNA, 26 bp, synthetic construct
  source 1..26: mol_type = other DNA
tctaaccctaactgagaagggcgtag

SEQ ID NO: 26 - DNA, 26 bp, synthetic construct
  source 1..26: mol_type = other DNA
gtttgctctagaatgaacggtggaag

SEQ ID NO: 27 - DNA, 19 bp, synthetic construct
  source 1..19: mol_type = other DNA
cgtgaagagctagtctctg

SEQ ID NO: 28 - DNA, 20 bp, synthetic construct
  source 1..20: mol_type = other DNA
ggttgtaggaactgagttcc

SEQ ID NO: 29 - DNA, 20 bp, synthetic construct
  source 1..20: mol_type = other DNA
ccagcttctggctcaaccac

SEQ ID NO: 30 - DNA, 22 bp, synthetic construct
  source 1..22: mol_type = other DNA
ccagaagagctatttggtagtg

SEQ ID NO: 31 - DNA, 20 bp, synthetic construct
  source 1..20: mol_type = other DNA
agaaagcatcggcaaaggtc

SEQ ID NO: 32 - DNA, 20 bp, synthetic construct
  source 1..20: mol_type = other DNA
cccaggatattttcatggcg

SEQ ID NO: 33 - DNA, 19 bp, synthetic construct
  source 1..19: mol_type = other DNA
caagggctcgctcagccag

SEQ ID NO: 34 - DNA, 20 bp, synthetic construct
  source 1..20: mol_type = other DNA
ccttggccacaatggtcttg

SEQ ID NO: 35 - DNA, 20 bp, synthetic construct
  source 1..20: mol_type = other DNA
ggcaagatgatcccaatgag

SEQ ID NO: 36 - DNA, 20 bp, synthetic construct
  source 1..20: mol_type = other DNA
ctgatctcacttggttctgg

SEQ ID NO: 37 - DNA, 20 bp, synthetic construct
  source 1..20: mol_type = other DNA
gccagagctgtgcagatgag

SEQ ID NO: 38 - DNA, 20 bp, synthetic construct
  source 1..20: mol_type = other DNA
cagtggacaggtttctgacc

SEQ ID NO: 39 - DNA, 22 bp, synthetic construct
  source 1..22: mol_type = other DNA
cctggagtttgtgaagaacaac

SEQ ID NO: 40 - DNA, 19 bp, synthetic construct
  source 1..19: mol_type = other DNA
ggtccttagccactccttc

SEQ ID NO: 41 - DNA, 18 bp, synthetic construct
  source 1..18: mol_type = other DNA
gagagaccctcactgctg

SEQ ID NO: 42 - DNA, 20 bp, synthetic construct
  source 1..20: mol_type = other DNA
gatggtacatgacaaggtgc

SEQ ID NO: 43 - DNA, 21 bp, synthetic construct
  source 1..21: mol_type = other DNA
gccaagtatgatgacatcaag

SEQ ID NO: 44 - DNA, 21 bp, synthetic construct
  source 1..21: mol_type = other DNA
gctgtagccatattcattgtc

SEQ ID NO: 45 - DNA, 36 bp, synthetic construct
  source 1..36: mol_type = other DNA
tcgacatgaatcttgacaagccctctaacccctgat

SEQ ID NO: 46 - DNA, 36 bp, synthetic construct
  source 1..36: mol_type = other DNA
ctagatcaggggttagagggcttgtcaagattcatg

SEQ ID NO: 47 - DNA, 48 bp, synthetic construct
  source 1..48: mol_type = other DNA
tcgacatgaatcttgacaagccctctaacccctcttcccatgagtgat

SEQ ID NO: 48 - DNA, 48 bp, synthetic construct
  source 1..48: mol_type = other DNA
ctagatcactcatgggaagaggggttagagggcttgtcaagattcatg

SEQ ID NO: 49 - DNA, 42 bp, synthetic construct
  source 1..42: mol_type = other DNA
tcgacatggacaagccctctaacccctcttcccatgagtgat

SEQ ID NO: 50 - DNA, 42 bp, synthetic construct
  source 1..42: mol_type = other DNA
ctagatcactcatgggaagaggggttagagggcttgtccatg

SEQ ID NO: 51 - DNA, 45 bp, synthetic construct
  source 1..45: mol_type = other DNA
tcgacatgcccaactctcccaaggaccttaatattttcggttgat

SEQ ID NO: 52 - DNA, 45 bp, synthetic construct
  source 1..45: mol_type = other DNA
ctagatcaaccgaaaatattaaggtccttgggagagttgggcatg

SEQ ID NO: 53 - DNA, 33 bp, synthetic construct
  source 1..33: mol_type = other DNA
tcgacatgggtttcattaatcttgacaagtgat

SEQ ID NO: 54 - DNA, 33 bp, synthetic construct
  source 1..33: mol_type = other DNA
ctagatcacttgtcaagattaatgaaacccatg

SEQ ID NO: 55 - DNA, 30 bp, synthetic construct
  source 1..30: mol_type = other DNA
tcgacatggacaagccctctaacccctgat

SEQ ID NO: 56 - DNA, 30 bp, synthetic construct
  source 1..30: mol_type = other DNA
ctagatcaggggttagagggcttgtccatg

SEQ ID NO: 57 - DNA, 42 bp, synthetic construct
  source 1..42: mol_type = other DNA
tcgacatggagcattcctctcccaactctcccaaggactgat

SEQ ID NO: 58 - RNA, 42 nt, synthetic construct
  source 1..42: mol_type = other RNA
ctagatcagtccttgggagagttgggagaggaatgctccatg

SEQ ID NO: 59 - DNA, 46 bp, synthetic construct
  source 1..46: mol_type = other DNA
tcgaccatgggtttcattaatcttgacaagccctctaacccctaag

SEQ ID NO: 60 - DNA, 46 bp, synthetic construct
  source 1..46: mol_type = other DNA
ctagacttaggggttagagggcttgtcaagattaatgaaacccatg

SEQ ID NO: 61 - DNA, 36 bp, synthetic construct
  source 1..36: mol_type = other DNA
atggacaagccctctaacccctcttcccatgagtga

SEQ ID NO: 62 - DNA, 7385 bp, synthetic construct
  source 1..7385: mol_type = other DNA
gtgtttaaacctagatattgatagtctgatcggtcaacgtataatcgagtcctagcttttgcaaacatctatcaagagacaggatcagcaggaggctttcgcatgattgaacaagatggattgcacgcaggttctccggcggcttgggtggagaggctattcggctatgactgggcacaacagacaatcggctgctctgatgccgccgtgttccggctgtcagcgcaggggcgtccggttctttttgtcaagaccgacctgtccggtgccctgaatgaactgcaagacgaggcagcgcggctatcgtggctggcgacgacgggcgttccttgcgcggctgtgctcgacgttgtcactgaagcgggaagggactggctgctattgggcgaagtgccggggcaggatctcctgtcatctcaccttgctcctgccgagaaagtatccatcatggctgatgcaatgcggcggctgcatacgcttgatccggctacctgcccattcgaccaccaagcgaaacatcgcatcgagcgagcacgtactcggatggaagccggtcttgtcgatcaggatgatctggacgaagagcatcaggggctcgcgccagccgaactgttcgccaggctcaaggcgtctatgcccgacggcgaggatctcgtcgtgacccacggcgatgcctgcttgccgaatatcatggtggaaaatggccgcttttctggattcatcgactgtggccgtctgggtgtggcggaccgctatcaggacatagcgttggctacccgtgatattgctgaagagcttggcggcgaatgggctgaccgcttccttgtgctttacggtatcgccgcgcccgattcgcagcgcatcgccttctatcgccttcttgacgagttcttctgaccgattctaggtgcattggcgcagaaaaaaatgcctgatgcgacgctgcgcgtcttatactcccacatatgccagattcagcaacggatacggcttccccaacttgcccacttccatacgtgtcctccttaccagaaatttatccttaacgatcggacggggagtcaggcaactatggatgaacgaaatagacagatcgctgagataggtgcctcactgattaagcattggtaactgtcagaccaagtttactcatatatactttagattgatttaaaacttcatttttaatttaaaaggatctaggtgaagatcctttttgataatctcatgaccaaaatcccttaacgtgagttttcgttccactgagcgtcagaccccgtagaaaagatcaaaggatcttcttgagatcctttttttctgcgcgtaatctgctgcttgcaaacaaaaaaaccaccgctaccagcggtggtttgtttgccggatcaagagctaccaactctttttccgaaggtaactggcttcagcagagcgcagataccaaatactgttcttctagtgtagccgtagttaggccaccacttcaagaactctgtagcaccgcctacatacctcgctctgctaatcctgttaccagtggctgctgccagtggcgataagtcgtgtcttaccgggttggactcaagacgatagttaccggataaggcgcagcggtcgggctgaacggggggttcgtgcacacagcccagcttggagcgaacgacctacaccgaactgagatacctacagcgtgagctatgagaaagcgccacgcttcccgaagggagaaaggcggacaggtatccggtaagcggcagggtcggaacaggagagcgcacgagggagcttccagggggaaacgcctggtatctttatagtcctgtcgggtttcgccacctctgacttgagcgtcgatttttgtgatgctcgtcaggggggcggagcctatggaaaaacgccagcaacgcggcctttttacggttcctggccttttgctggccttttgctcacatgttctttcctgcgttatcccctgattctgtggataaccgtattaccgcctttgagtgagctgataccgctcgccgcagccgaacgaccgagcgcagcgagtcagtgagcgaggaagcggaagagcgcccaatacgcaaaccgcctctccccgcgcgttggccgattcattaatgcagctggcacgacaggtttcccgactggaaagcgggcagtgagcgcaacgcaattaatgtgagttagctcactcattaggcaccccaggctttacactttatgcttccggctcgtatgttgtgtggaattgtgagcggataacaatttcacacaggaaacagctatgaccatgattacgccaagcgcgcaattaaccctcactaaagggaacaaaagctggagctgcaagcttggccattgcatacgttgtatccatatcataatatgtacatttatattggctcatgtccaacattaccgccatgttgacattgattattgactagttattaatagtaatcaattacggggtcattagttcatagcccatatatggagttccgcgttacataacttacggtaaatggcccgcctggctgaccgcccaacgacccccgcccattgacgtcaataatgacgtatgttcccatagtaacgccaatagggactttccattgacgtcaatgggtggagtatttacggtaaactgcccacttggcagtacatcaagtgtatcatatgccaagtacgccccctattgacgtcaatgacggtaaatggcccgcctggcattatgcccagtacatgaccttatgggactttcctacttggcagtacatctacgtattagtcatcgctattaccatggtgatgcggttttggcagtacatcaatgggcgtggatagcggtttgactcacggggatttccaagtctccaccccattgacgtcaatgggagtttgttttggcaccaaaatcaacgggactttccaaaatgtcgtaacaactccgccccattgacgcaaatgggcggtaggcgtgtacggtgggaggtctatataagcagagctcgtttagtgaaccggggtctctctggttagaccagatctgagcctgggagctctctggctaactagggaacccactgcttaagcctcaataaagcttgccttgagtgcttcaagtagtgtgtgcccgtctgttgtgtgactctggtaactagagatccctcagacccttttagtcagtgtggaaaatctctagcagtggcgcccgaacagggacttgaaagcgaaagggaaaccagaggagctctctcgacgcaggactcggcttgctgaagcgcgcacggcaagaggcgaggggcggcgactggtgagtacgccaaaaattttgactagcggaggctagaaggagagagatgggtgcgagagcgtcagtattaagcgggggagaattagatcgcgatgggaaaaaattcggttaaggccagggggaaagaaaaaatataaattaaaacatatagtatgggcaagcagggagctagaacgattcgcagttaatcctggcctgttagaaacatcagaaggctgtagacaaatactgggacagctacaaccatcccttcagacaggatcagaagaacttagatcattatataatacagtagcaaccctctattgtgtgcatcaaaggatagagataaaagacaccaaggaagctttagacaagatagaggaagagcaaaacaaaagtaagaccaccgcacagcaagcggccgctgatcttcagacctggaggaggagatatgagggacaattggagaagtgaattatataaatataaagtagtaaaaattgaaccattaggagtagcacccaccaaggcaaagagaagagtggtgcagagagaaaaaagagcagtgggaataggagctttgttccttgggttcttgggagcagcaggaagcactatgggcgcagcgtcaatgacgctgacggtacaggccagacaattattgtctggtatagtgcagcagcagaacaatttgctgagggctattgaggcgcaacagcatctgttgcaactcacagtctggggcatcaagcagctccaggcaagaatcctggctgtggaaagatacctaaaggatcaacagctcctggggatttggggttgctctggaaaactcatttgcaccactgctgtgccttggaatgctagttggagtaataaatctctggaacagatttggaatcacacgacctggatggagtgggacagagaaattaacaattacacaagcttaatacactccttaattgaagaatcgcaaaaccagcaagaaaagaatgaacaagaattattggaattagataaatgggcaagtttgtggaattggtttaacataacaaattggctgtggtatataaaattattcataatgatagtaggaggcttggtaggtttaagaatagtttttgctgtactttctatagtgaatagagttaggcagggatattcaccattatcgtttcagacccacctcccaaccccgaggggacccgacaggcccgaaggaatagaagaagaaggtggagagagagacagagacagatccattcgattagtgaacggatctcgacggtatcggttaacttttaaaagaaaaggggggattggggggtacagtgcaggggaaagaatagtagacataatagcaacagacatacaaactaaagaattacaaaaacaaattacaaaaattcaaaattttatcgatcacgagactagcctcgagaagcttgatatcgaattccacggggttggggttgcgccttttccaaggcagccctgggtttgcgcagggacgcggctgctctgggcgtggttccgggaaacgcagcggcgccgaccctgggtctcgcacattcttcacgtccgttcgcagcgtcacccggatcttcgccgctacccttgtgggccccccggcgacgcttcctgctccgcccctaagtcgggaaggttccttgcggttcgcggcgtgccggacgtgacaaacggaagccgcacgtctcactagtaccctcgcagacggacagcgccagggagcaatggcagcgcgccgaccgcgatgggctgtggccaatagcggctgctcagcagggcgcgccgagagcagcggccgggaaggggcggtgcgggaggcggggtgtggggcggtagtgtgggccctgttcctgcccgcgcggtgttccgcattctgcaagcctccggagcgcacgtcggcagtcggctccctcgttgaccgaatcaccgacctctctccccagggggatccgtcgaccatgggtttcattaatcttgacaagccctctaacccctaagtctagaggatcccccgggctgcaggaattcgagcatcttaccgccatttattcccatatttgttctgtttttcttgatttgggtatacatttaaatgttaataaaacaaaatggtggggcaatcatttacatttttagggatatgtaattactagttcaggtgtattgccacaagacaaacatgttaagaaactttcccgttatttacgctctgttcctgttaatcaacctctggattacaaaatttgtgaaagattgactgatattcttaactatgttgctccttttacgctgtgtggatatgctgctttaatgcctctgtatcatgctattgcttcccgtacggctttcgttttctcctccttgtataaatcctggttgctgtctctttatgaggagttgtggcccgttgtccgtcaacgtggcgtggtgtgctctgtgtttgctgacgcaacccccactggctggggcattgccaccacctgtcaactcctttctgggactttcgctttccccctcccgatcgccacggcagaactcatcgccgcctgccttgcccgctgctggacaggggctaggttgctgggcactgataattccgtggtgttgtcggggaagggcctgctgccggctctgcggcctcttccgcgtcttcgccttcgccctcagacgagtcggatctccctttgggccgcctccccgcctggaattcgagctcggtacctttaagaccaatgacttacaaggcagctgtagatcttagccactttttaaaagaaaaggggggactggaagggctaattcactcccaacgaagacaagatctgctttttgcttgtactgggtctctctggttagaccagatctgagcctgggagctctctggctaactagggaacccactgcttaagcctcaataaagcttgccttgagtgcttcaagtagtgtgtgcccgtctgttgtgtgactctggtaactagagatccctcagacccttttagtcagtgtggaaaatctctagcagtagtagttcatgtcatcttattattcagtatttataacttgcaaagaaatgaatatcagagagtgagaggaacttgtttattgcagcttataatggttacaaataaagcaatagcatcacaaatttcacaaataaagcatttttttcactgcattctagttgtggtttgtccaaactcatcaatgtatcttatcatgtctggctctagctatcccgcccctaactccgcccatcccgcccctaactccgcccagttccgcccattctccgccccatggctgactaattttttttatttatgcagaggccgaggccgcctcggcctctgagctattccagaagtagtgaggaggcttttttggaggcctagggacgtacccaattcgccctatagtgagtcgtattacgcgcgctcactggccgtcgttttacaacgtcgtgactgggaaaaccctggcgttacccaacttaatcgccttgcagcacatccccctttcgccagctggcgtaatagcgaagaggcccgcaccgatcgcccttcccaacagttgcgcagcctgaatggcgaatgggacgcgccctgtagcggcgcattaagcgcggcgggtgtggtggttacgcgcagcgtgaccgctacacttgccagcgccctagcgcccgctcctttcgctttcttcccttcctttctcgccacgttcgccggctttccccgtcaagctctaaatcgggggctccctttagggttccgatttagtgctttacggcacctcgaccccaaaaaacttgattagggtgatggttcacgtagtgggccatcgccctgatagacggtttttcgccctttgacgttggagtccacgttctttaatagtggactcttgttccaaactggaacaacactcaaccctatctcggtctattcttttgatttataagggattttgccgatttcggcctattggttaaaaaatgagctgatttaacaaaaatttaacgcgaattttaacaaaatcgttccctcaggacgtc

SEQ ID NO: 63 - DNA, 7377 bp, synthetic construct
  source 1..7377: mol_type = other DNA
caggtggcacttttcggggaaatgtgcgcggaacccctatttgtttatttttctaaatacattcaaatatgtatccgctcatgagacaataaccctgataaatgcttcaataatattgaaaaaggaagagtatgagtattcaacatttccgtgtcgcccttattcccttttttgcggcattttgccttcctgtttttgctcacccagaaacgctggtgaaagtaaaagatgctgaagatcagttgggtgcacgagtgggttacatcgaactggatctcaacagcggtaagatccttgagagttttcgccccgaagaacgttttccaatgatgagcacttttaaagttctgctatgtggcgcggtattatcccgtattgacgccgggcaagagcaactcggtcgccgcatacactattctcagaatgacttggttgagtactcaccagtcacagaaaagcatcttacggatggcatgacagtaagagaattatgcagtgctgccataaccatgagtgataacactgcggccaacttacttctgacaacgatcggaggaccgaaggagctaaccgcttttttgcacaacatgggggatcatgtaactcgccttgatcgttgggaaccggagctgaatgaagccataccaaacgacgagcgtgacaccacgatgcctgtagcaatggcaacaacgttgcgcaaactattaactggcgaactacttactctagcttcccggcaacaattaatagactggatggaggcggataaagttgcaggaccacttctgcgctcggcccttccggctggctggtttattgctgataaatctggagccggtgagcgtgggtctcgcggtatcattgcagcactggggccagatggtaagccctcccgtatcgtagttatctacacgacggggagtcaggcaactatggatgaacgaaatagacagatcgctgagataggtgcctcactgattaagcattggtaactgtcagaccaagtttactcatatatacttagattgatttaaaacttcatttttaatttaaaaggatctaggtgaagatcctttttgataatctcatgaccaaaatcccttaacgtgagttttcgttccactgagcgtcagaccccgtagaaaagatcaaaggatcttcttgagatcctttttttctgcgcgtaatctgctgcttgcaaacaaaaaaaccaccgctaccagcggtggtttgtttgccggatcaagagctaccaactctttttccgaaggtaactggcttcagcagagcgcagataccaaatactgtccttctagtgtagccgtagttaggccaccacttcaagaactctgtagcaccgcctacatacctcgctctgctaatcctgttaccagtggctgctgccagtggcgataagtcgtgtcttaccgggttggactcaagacgatagttaccggataaggcgcagcggtcgggctgaacggggggttcgtgcacacagcccagcttggagcgaacgacctacaccgaactgagatacctacagcgtgagctatgagaaagcgccacgcttcccgaagggagaaaggcggacaggtatccggtaagcggcagggtcggaacaggagagcgcacgagggagcttccagggggaaacgcctggtatctttatagtcctgtcgggtttcgccacctctgacttgagcgtcgatttttgtgatgctcgtcaggggggcggagcctatggaaaaacgccagcaacgcggcctttttacggttcctggccttttgctggccttttgctcacatgttctttcctgcgttatcccctgattctgtggataaccgtattaccgcctttgagtgagctgataccgctcgccgcagccgaacgaccgagcgcagcgagtcagtgagcgaggaagcggaagagcgcccaatacgcaaaccgcctctccccgcgcgttggccgattcattaatgcagctggcacgacaggtttcccgactggaaagcgggcagtgagcgcaacgcaattaatgtggttagctcactcattaggcaccccaggctttacactttatgcttccggctcgtatgttgtgtggaattgtgagcggataacaatttcacacaggaaacagctatgaccatgattacgccaagcgcgcaattaaccctcactaaagggaacaaaagctggagctgcaagcttaatgtagtcttatgcaatactcttgtagtcttgcaacatggtaacgatgagttagcaacatgccttacaaggagagaaaaagcaccgtgcatgccgattggtggaagtaaggtggtacgatcgtgccttattaggaaggcaacagacgggtctgacatggattggacgaaccactgaattgccgcattgcagagatattgtatttaagtgcctagctcgatacaataaacgggtctctctggttagaccagatctgagcctgggagctctctggctaactagggaacccactgcttaagcctcaataaagcttgccttgagtgcttcaagtagtgtgtgcccgtctgttgtgtgactctggtaactagagatccctcagacccttttagtcagtgtggaaaatctctagcagtggcgcccgaacagggacctgaaagcgaaagggaaaccagagctctctcgacgcaggactcggcttgctgaagcgcgcacggcaagaggcgaggggcggcgactggtgagtacgccaaaaattttgactagcggaggctagaaggagagagatgggtgcgagagcgtcagtattaagcgggggagaattagatcgcgatgggaaaaaattcggttaaggccagggggaaagaaaaaatataaattaaaacatatagtatgggcaagcagggagctagaacgattcgcagttaatcctggcctgttagaaacatcagaaggctgtagacaaatactgggacagctacaaccatcccttcagacaggatcagaagaacttagatcattatataatacagtagcaaccctctattgtgtgcatcaaaggatagagataaaagcaccaaggaagctttagacaagatagaggaagagcaaaacaaaagtaagaccaccgcacagcaagcggccgctgatcttcagacctggaggaggagatatgagggacaattggagaagtgaattatataaatataaagtagtaaaaattgaaccattaggagtagcacccaccaaggcaaagagaagagtggtgcagagagaaaaaagagcagtgggaataggagctttgttccttgggttcttgggagcagcaggaagcactatgggcgcagcctcaatgacgctgacggtacaggccagacaattattgtctggtatagtgcagcagcagaacaatttgctgagggctattgaggcgcaacagcatctgttgcaactcacagtctggggcatcaagcagctccaggcaagaatcctggctgtggaaagatacctaaaggatcaacagctcctggggatttggggttgctctggaaaactcatttgcaccactgctgtgccttggaatgctagttggagtaataaatctctggaacagatttggaatcacacgacctggatggagtgggacagagaaattaacaattacacaagcttaatacactccttaattgaagaatcgcaaaaccagcaagaaaagaatgaacaagaattattggaattagataaatgggcaagtttgtggaattggtttaacataacaaattggctgtggtatataaaattattcataatgatagtaggaggcttggtaggtttaagaatagtttttgctgtactttctatagtgaatagagttaggcagggatattcaccattatcgtttcagacccacctcccaaccccgaggggacccgacaggcccgaaggaatagaagaagaaggtggagagagagacagagacagatccattcgattagtgaacggatctcgacggtatcggttaacttttaaaagaaaaggggggattggggggtacagtgcaggggaaagaatagtagacataatagcaacagacataaaactaaagaattacaaaaacaaattacaaaaattcaaaattttatcgatcacgagactagcctcgagaagcttgatatcgaattcccacggggttggggttgcgccttttccaaggcagccctgggtttgcgcagggacgcggctgctctgggcgtggttccgggaaacgcagcggcgccgaccctgggtctcgcacattcttcacgtccgttcgcagcgtcacccggatcttcgccgctacccttgtgggccccccggcgacgcttcctgctccgcccctaagtcgggaaggttccttgcggttcgcggcgtgccggacgtgacaaacggaagccgcacgtctcactagtaccctcgcagacggacagcgccagggagcaatggcagcgcgccgaccgcgatgggctgtggccaatagcggctgctcagcggggcgcgccgagagcagcggccgggaaggggcggtgcgggaggcggggtgtggggcggtagtgtgggccctgttcctgcccgcgcggtgttccgcattctgcaagcctccggagcgcacgtcggcagtcggctccctcgttgaccgaatcaccgacctctctccccagggggatccaccggtcgccaccatggtgagcaagggcgaggagctgttcaccggggtggtgcccatcctggtcgagctggacggcgacgtaaacggccacaagttcagcgtgtccggcgagggcgagggcgatgccacctacggcaagctgaccctgaagttcatctgcaccaccggcaagctgcccgtgccctggcccaccctcgtgaccaccctgacctacggcgtgcagtgcttcagccgctaccccgaccacatgaagcagcacgacttcttcaagtccgccatgcccgaaggctacgtccaggagcgcaccatcttcttcaaggacgacggcaactacaagacccgcgccgaggtgaagttcgagggcgacaccctggtgaaccgcatcgagctgaagggcatcgacttcaaggaggcggcaacatcctggggcacaagctggagtacaactacaacagccacaacgtctatatcatggccgacaagcagaagaacggcatcaaggtgaacttcaagatccgccacaacatcgaggacggcagcgtgcagctcgccgaccactaccagcagaacacccccatcggcgacggccccgtgctgctgcccgacaaccactacctgagcacccagtccgccctgagcaaagaccccaacgagaagcgcgatcacatggtcctgctggagttcgtgaccgccgccgggatcactctcggcatggacgagctgtacaagtaaagcggccgcgtcgacaatcaacctctggattacaaaatttgtgaaagattgactggtattcttaactatgttgctccttttacgctatgtggatacgctgctttaatgcctttgtatcatgctattgcttcccgtatggctttcattttctcctccttgtataaatcctggttgctgtctctttatgaggagttgtggcccgttgtcaggcaacgtggcgtggtgtgcactgtgtttgctgacgcaacccccactggttggggcattgccaccacctgtcagctcctttccgggactttcgctttccccctccctattgccacggcggaactcatcgccgcctgccttgcccgctgctggacaggggctcggctgttgggcactgacaattccgtggtgttgtcggggaagctgacgtcctttccatggctgctcgcctgtgttgccacctggattctgcgcgggacgtccttctgctacgtcccttcggccctcaatccagcggaccttccttcccgcggcctgctgccggctctgcggcctcttccgcgtcttcgccttcgccctcagacgagtcggatctccctttgggccgcctccccgcctggaattcgagctcggtacctttaagaccaatgacttacaaggcagctgtagatcttagccactttttaaaagaaaaggggggactggaagggctaatcactcccaacgaagacaagatctgctttttgcttgtactgggtctctctggttagaccagatctgagcctgggagctctctggctaactagggaacccactgcttaagcctcaataaagcttgccttgagtgcttcaagtagtgtgtgcccgtctgttgtgtgactctggtaactagagatccctcagacccttttagtcagtgtggaaaatctctagcagtagtagttcatgtcatcttattattcagtatttataacttgcaaagaaatgaatatcagagagtgagaggaacttgtttattgcagcttataatggttacaaataaagcaatagcatcacaaatttcacaaataaagcatttttttcactgcattctagttgtggtttgtccaaactcatcaatgtatcttatcatgtctggctctagctatcccgcccctaactccgcccagttccgcccattctccgccccatggctgactaattttttttatttatgcagaggccgaggccgcctcggcctctgagctattccagaagtagtgaggaggcttttttggaggcctaggcttttgcgtcgagacgtacccaattcgccctatagtgagtcgtattacgcgcgctcactggccgtcgttttacaacgtcgtgactgggaaaaccctggcgttacccaacttaatcgccttgcagcacatccccctttcgccagctggcgtaatagcgaagaggcccgcaccgatcgcccttcccaacagttgcgcagcctgaatggcgaatggcgcgacgcgccctgtagcggcgcattaagcgcggcgggtgtggtggttacgcgcagcgtgaccgctacacttgccagcgccctagcgcccgctcctttcgctttcttcccttcctttctcgccacgttcgccggctttccccgtcaagctctaaatcgggggctccctttagggttccgatttagtgctttacggcacctcgaccccaaaaaacttgattagggtgatggttcacgtatgggccatcgccctgatagacggtttttcgccctttgacgttggagtccacgttctttaatagtggactcttgttccaaactggaacaacactcaaccctatctcggtctattcttttgatttataagggattttgccgatttcggcctattggttaaaaaatgagctgatttaacaaaaatttaacgcgaattttaacaaaatattaacgtttacaatttcc

SEQ ID NO: 64 - protein, 514 aa, Homo sapiens
MADAEVIILPKKHKKKKERKSLPEEDVAEIQHAEEFLIKPESKVAKLDTSQWPLLLKNFDKLNVRTTHYTPLACGSNPLKREIGDYIRTGFINLDKPSNPSSHEVVAWIRRILRVEKTGHSGTLDPKVTGCLIVCIERATRLVKSQQSAGKEYVGIVRLHNAIEGGTQLSRALETLTGALFQRPPLIAAVKRQLRVRTIYESKMIEYDPERRLGIFWVSCEAGTYIRTLCVHLGLLLGVGGQMQELRRVRSGVMSEKDHMVTMHDVLDAQWLYDNHKDESYLRRVVYPLEKLLTSHKRLVMKDSAVNAICYGAKIMLPGVLRYEDGIEVNQEIVVITTKGEAICMAIALMTTAVISTCDHGIVAKIKRVIMERDTYPRKWGLGPKASQKKLMIKQGLLDKHGKPTDSTPATWKQEYVDYSESAKKEVVAEVVKAPQVVAEAAKTAKRKRESESESDETPPAAPQLIKKEKKKSKKDKKAKAGLESGAEPGDGDSDTTKKKKKKKKAKEVELVSE